European Patent Application EP 4 574 979 A1, published June 25, 2025. Title: ENGINEERED IMMUNE CELL AND PREPARATION METHOD THEREFOR. Applicant: CELLS & GENES BIOTECH (SHANGHAI) CO., LTD. The sequence listing filed with the application follows.

SEQUENCE LISTING (32 sequences)

SEQ ID NO: 1 - protein, 242 aa, synthetic construct
  source 1..242: note = target-binding domain of GPC3-CAR
QVQLVQSGAEVKKPGASVKVSCKASGYTFTDYEMHWVRQAPGQGLEWMGALDPKTGDTAYSQKFKGRVTLTADKSTSTAYMELSSLTSEDTAVYYCTRFYSYTYWGQGTLVTVSSGGGGSGGGGSGGGGSDVVMTQSPLSLPVTPGEPASISCRSSQSLVHSNGNTYLHWYLQKPGQSPQLLIYKVSNRFSGVPDRFSGSGSGTDFTLKISRVEAEDVGVYYCSQNTHVPPTFGQGTKLEIK

SEQ ID NO: 2 - protein, 69 aa, synthetic construct
  source 1..69: note = CD8 alpha hinge and transmembrane domains
TTTPAPRPPTPAPTIASQPLSLRPEACRPAAGGAVHTRGLDFACDIYIWAPLAGTCGVLLLSLVITLYC

SEQ ID NO: 3 - protein, 42 aa, synthetic construct
  source 1..42: note = 41BB co-stimulatory domain
KRGRKKLLYIFKQPFMRPVQTTQEEDGCSCRFPEEEEGGCEL

SEQ ID NO: 4 - protein, 112 aa, synthetic construct
  source 1..112: note = CD3 zeta
RVKFSRSADAPAYQQGQNQLYNELNLGRREEYDVLDKRRGRDPEMGGKPRRKNPQEGLYNELQKDKMAEAYSEIGMKGERRRGKGHDGLYQGLSTATKDTYDALHMQALPPR

SEQ ID NO: 5 - protein, 486 aa, synthetic construct
  source 1..486: note = GPC3-CAR
MALPVTALLLPLALLLHAARPQVQLVQSGAEVKKPGASVKVSCKASGYTFTDYEMHWVRQAPGQGLEWMGALDPKTGDTAYSQKFKGRVTLTADKSTSTAYMELSSLTSEDTAVYYCTRFYSYTYWGQGTLVTVSSGGGGSGGGGSGGGGSDVVMTQSPLSLPVTPGEPASISCRSSQSLVHSNGNTYLHWYLQKPGQSPQLLIYKVSNRFSGVPDRFSGSGSGTDFTLKISRVEAEDVGVYYCSQNTHVPPTFGQGTKLEIKTTTPAPRPPTPAPTIASQPLSLRPEACRPAAGGAVHTRGLDFACDIYIWAPLAGTCGVLLLSLVITLYCKRGRKKLLYIFKQPFMRPVQTTQEEDGCSCRFPEEEEGGCELRVKFSRSADAPAYQQGQNQLYNELNLGRREEYDVLDKRRGRDPEMGGKPRRKNPQEGLYNELQKDKMAEAYSEIGMKGERRRGKGHDGLYQGLSTATKDTYDALHMQALPPR

SEQ ID NO: 6 - protein, 114 aa, Homo sapiens
NWVNVISDLKKIEDLIQSMHIDATLYTESDVHPSCKVTAMKCFLLELQVISLESGDASIHDTVENLIILANNSLSSNGNVTESGCKECEELEEKNIKEFLQSFVHIVQMFINTS

SEQ ID NO: 7 - protein, 162 aa, Homo sapiens
MRISKPHLRSISIQCYLCLLLNSHFLTEAGIHVFILGCFSAGLPKTEANWVNVISDLKKIEDLIQSMHIDATLYTESDVHPSCKVTAMKCFLLELQVISLESGDASIHDTVENLIILANNSLSSNGNVTESGCKECEELEEKNIKEFLQSFVHIVQMFINTS

SEQ ID NO: 8 - protein, 25 aa, synthetic construct
  source 1..25: note = IL-7 signal peptide
MFHVSFRYIFGLPPLILVLLPVASS

SEQ ID NO: 9 - protein, 139 aa, synthetic construct
  source 1..139: note = IL-7-IL15
MFHVSFRYIFGLPPLILVLLPVASSNWVNVISDLKKIEDLIQSMHIDATLYTESDVHPSCKVTAMKCFLLELQVISLESGDASIHDTVENLIILANNSLSSNGNVTESGCKECEELEEKNIKEFLQSFVHIVQMFINTS

SEQ ID NO: 10 - protein, 131 aa, Homo sapiens
QDRHMIRMRQLIDIVDQLKNYVNDLVPEFLPAPEDVETNCEWSAFSCFQKAQLKSANTGNNERIINVSIKKLKRKPPSTNAGRRQKHRLTCPSCDSYEKKPPKEFLERFKSLLQKMIHQHLSSRTHGSEDS

SEQ ID NO: 11 - protein, 162 aa, Homo sapiens
MRSSPGNMERIVICLMVIFLGTLVHKSSSQGQDRHMIRMRQLIDIVDQLKNYVNDLVPEFLPAPEDVETNCEWSAFSCFQKAQLKSANTGNNERIINVSIKKLKRKPPSTNAGRRQKHRLTCPSCDSYEKKPPKEFLERFKSLLQKMIHQHLSSRTHGSEDS

SEQ ID NO: 12 - protein, 21 aa, synthetic construct
  source 1..21: note = CD19 signal peptide
MALLLALSLLVLWTSPAPTLS

SEQ ID NO: 13 - protein, 152 aa, synthetic construct
  source 1..152: note = CCL19-IL-21
MALLLALSLLVLWTSPAPTLSQDRHMIRMRQLIDIVDQLKNYVNDLVPEFLPAPEDVETNCEWSAFSCFQKAQLKSANTGNNERIINVSIKKLKRKPPSTNAGRRQKHRLTCPSCDSYEKKPPKEFLERFKSLLQKMIHQHLSSRTHGSEDS

SEQ ID NO: 14 - protein, 18 aa, synthetic construct
  source 1..18: note = T2A
EGRGSLLTCGDVEENPGP

SEQ ID NO: 15 - protein, 22 aa, synthetic construct
  source 1..22: note = P2A
GSGATNFSLLKQAGDVEENPGP

SEQ ID NO: 16 - protein, 25 aa, synthetic construct
  source 1..25: note = F2A
GSGVKQTLNFDLLKLAGDVESNPGP

SEQ ID NO: 17 - DNA, 400 bp, synthetic construct
  source 1..400: mol_type = other DNA; note = 5' homologous arm
cagtttgctttgctgggcctttttcccatgcctgcctttactctgccagagttatattgctggggttttgaagaagatcctattaaataaaagaataagcagtattattaagtagccctgcatttcaggtttccttgagtggcaggccaggcctggccgtgaacgttcactgaaatcatggcctcttggccaagattgatagcttgtgcctgtccctgagtcccagtccatcacgagcagctggtttctaagatgctatttcccgtataaagcatgagaccgtgacttgccagccccacagagccccgcccttgtccatcactggcatctggactccagcctgggttggggcaaagagggaaatgagatcatgtcctaaccctgatcctcttgtcccaca

SEQ ID NO: 18 - DNA, 400 bp, synthetic construct
  source 1..400: mol_type = other DNA; note = 3' homologous arm
gatatccagaaccctgaccctgccgtgtaccagctgagagactctaaatccagtgacaagtctgtctgcctattcaccgattttgattctcaaacaaatgtgtcacaaagtaaggattctgatgtgtatatcacagacaaaactgtgctagacatgaggtctatggacttcaagagcaacagtgctgtggcctggagcaacaaatctgactttgcatgtgcaaacgccttcaacaacagcattattccagaagacaccttcttccccagcccaggtaagggcagctttggtgccttcgcaggctgtttccttgcttcaggaatggccaggttctgcccagagctctggtcaatgatgtctaaaactcctctgattggtggtctcggccttatccattgcc

SEQ ID NO: 19 - protein, 857 aa, synthetic construct
  source 1..857: note = GPC3CAR-2A-IL15-2A-IL-21
MALPVTALLLPLALLLHAARPQVQLVQSGAEVKKPGASVKVSCKASGYTFTDYEMHWVRQAPGQGLEWMGALDPKTGDTAYSQKFKGRVTLTADKSTSTAYMELSSLTSEDTAVYYCTRFYSYTYWGQGTLVTVSSGGGGSGGGGSGGGGSDVVMTQSPLSLPVTPGEPASISCRSSQSLVHSNGNTYLHWYLQKPGQSPQLLIYKVSNRFSGVPDRFSGSGSGTDFTLKISRVEAEDVGVYYCSQNTHVPPTFGQGTKLEIKTTTPAPRPPTPAPTIASQPLSLRPEACRPAAGGAVHTRGLDFACDIYIWAPLAGTCGVLLLSLVITLYCKRGRKKLLYIFKQPFMRPVQTTQEEDGCSCRFPEEEEGGCELRVKFSRSADAPAYQQGQNQLYNELNLGRREEYDVLDKRRGRDPEMGGKPRRKNPQEGLYNELQKDKMAEAYSEIGMKGERRRGKGHDGLYQGLSTATKDTYDALHMQALPPRGSGATNFSLLKQAGDVEENPGPMRISKPHLRSISIQCYLCLLLNSHFLTEAGIHVFILGCFSAGLPKTEANWVNVISDLKKIEDLIQSMHIDATLYTESDVHPSCKVTAMKCFLLELQVISLESGDASIHDTVENLIILANNSLSSNGNVTESGCKECEELEEKNIKEFLQSFVHIVQMFINTSGSGVKQTLNFDLLKLAGDVESNPGPMRSSPGNMERIVICLMVIFLGTLVHKSSSQGQDRHMIRMRQLIDIVDQLKNYVNDLVPEFLPAPEDVETNCEWSAFSCFQKAQLKSANTGNNERIINVSIKKLKRKPPSTNAGRRQKHRLTCPSCDSYEKKPPKEFLERFKSLLQKMIHQHLSSRTHGSEDS

SEQ ID NO: 20 - DNA, 2845 bp, synthetic construct
  source 1..2845: mol_type = other DNA; note = GPC3CAR-2A-IL15-2A-IL-21
atggccttaccagtgaccgccttgctcctgccgctggccttgctgctccacgccgccaggccgcaggtgcagctggtgcagtctggagctgaggtgaagaagcctggggcctcagtgaaggtctcctgcaaggcttctggatacaccttcaccgactatgaaatgcactgggtgcgacaggcccctggacaagggcttgagtggatgggagctcttgatcctaaaactggtgatactgcctacagtcagaagttcaagggcagagtcacgctgaccgcggacaaatccacgagcacagcctacatggagctgagcagcctgacatctgaggacacggccgtgtattactgtacaagattctactcctatacttactggggccagggaaccctggtcaccgtctcctcaggaggaggaggctctggaggaggagggagtggaggcgggggaagcgacgtggtgatgacccagagccccctgagcctgcccgtgacccccggcgagcccgccagcatcagctgcaggagcagccagagcctggtgcacagcaacggcaacacctacctgcactggtacctgcagaagcccggccagagcccccagctgctgatctacaaggtgagcaacaggttcagcggcgtgcccgacaggttcagcggcagcggcagcggcaccgacttcaccctgaagatcagcagggtggaggccgaggacgtgggcgtgtactactgcagccagaacacccacgtgccccccaccttcggccagggcaccaagctggagatcaagaccacgacgccagcgccgcgaccaccaacaccggcgcccaccatcgcgtcgcagcccctgtccctgcgcccagaggcgtgccggccagcggcggggggcgcagtgcacacgagggggctggacttcgcctgtgatatctacatctgggcgcccttggccgggacttgtggggtccttctcctgtcactggttatcaccctttactgcaaacggggcagaaagaaactcctgtatatattcaaacaaccatttatgagaccagtacaaactactcaagaggaagatggctgtagctgccgatttccagaagaagaagaaggaggatgtgaactgagagtgaagttcagcaggagcgcagacgcccccgcgtaccagcagggccagaaccagctctataacgagctcaatctaggacgaagagaggagtacgatgttttggacaagagacgtggccgggaccctgagatggggggaaagccgagaaggaagaaccctcaggaaggcctgtacaatgaactgcagaaagataagatggcggaggcctacagtgagattgggatgaaaggcgagcgccggaggggcaaggggcacgatggcctttaccagggtctcagtacagccaccaaggacacctacgacgcccttcacatgcaggccctgccccctcgcggcagcggcgccacaaacttctctctgctaaagcaagcaggtgatgttgaagaaaaccccgggcctatgagaatttcgaaaccacatttgagaagtatttccatccagtgctacttgtgtttacttctaaacagtcattttctaactgaagctggcattcatgtcttcattttgggctgtttcagtgcagggcttcctaaaacagaagccaactgggtgaatgtaataagtgatttgaaaaaaattgaagatcttattcaatctatgcatattgatgctactttatatacggaaagtgatgttcaccccagttgcaaagtaacagcaatgaagtgctttctcttggagttacaagttatttcacttgagtccggagatgcaagtattcatgatacagtagaaaatctgatcatcctagcaaacaacagtttgtcttctaatgggaatgtaacagaatctggatgcaaagaatgtgaggaactggaggaaaaaaatattaaagaatttttgcagagttttgtacatattgtccaaatgttcatcaacacttctggttctggcgtgaaacagactttgaattttgaccttctcaagttggcgggagacgtggagtccaacccagggcccatgagatccagtcctggcaacatggagaggattgtcatctgtctgatggtcatcttcttggggacactggtccacaaatcaagctcccaaggtcaagatcgccacatgattagaatgcgtcaacttatagatattgttgatcagctgaaaaattatgtgaatgacttggtccctgaatttctgccagctccagaagatgtagagacaaactgtgagtggtcagctttttcctgctttcagaaggcccaactaaagtcagcaaatacaggaaacaatgaaaggataatcaatgtatcaattaaaaagctgaagaggaaaccaccttccacaaatgcagggagaagacagaaacacagactaacatgcccttcatgtgattcttatgagaaaaaaccacccaaagaattcctagaaagattcaaatcacttctccaaaagatgattcatcagcatctgtcctctagaacacacggaagtgaagattcctgactgtgccttctagttgccagccatctgttgtttgcccctcccccgtgccttccttgaccctggaaggtgccactcccactgtcctttcctaataaaatgaggaaattgcatcgcattgtctgagtaggtgtcattctattctggggggtggggtggggcaggacagcaagggggaggattgggaagacaatagcaggcatgctggggatgcggtgggctctatgggaattctctagaaatattctcgaggtttaaacgtcgacgcggccgc

SEQ ID NO: 21 - DNA, 3757 bp, synthetic construct
  source 1..3757: mol_type = other DNA; note = GPC3CAR-2A-IL15-2A-IL-21 with homologous arms
cagtttgctttgctgggcctttttcccatgcctgcctttactctgccagagttatattgctggggttttgaagaagatcctattaaataaaagaataagcagtattattaagtagccctgcatttcaggtttccttgagtggcaggccaggcctggccgtgaacgttcactgaaatcatggcctcttggccaagattgatagcttgtgcctgtccctgagtcccagtccatcacgagcagctggtttctaagatgctatttcccgtataaagcatgagaccgtgacttgccagccccacagagccccgcccttgtccatcactggcatctggactccagcctgggttggggcaaagagggaaatgagatcatgtcctaaccctgatcctcttgtcccacactgacctcttctcttcctcccacagggcctcgagagatctggcagcggagagggcagaggaagtcttctaacatgcggtgacgtggaggagaatcccggccctaggctcgagatggccttaccagtgaccgccttgctcctgccgctggccttgctgctccacgccgccaggccgcaggtgcagctggtgcagtctggagctgaggtgaagaagcctggggcctcagtgaaggtctcctgcaaggcttctggatacaccttcaccgactatgaaatgcactgggtgcgacaggcccctggacaagggcttgagtggatgggagctcttgatcctaaaactggtgatactgcctacagtcagaagttcaagggcagagtcacgctgaccgcggacaaatccacgagcacagcctacatggagctgagcagcctgacatctgaggacacggccgtgtattactgtacaagattctactcctatacttactggggccagggaaccctggtcaccgtctcctcaggaggaggaggctctggaggaggagggagtggaggcgggggaagcgacgtggtgatgacccagagccccctgagcctgcccgtgacccccggcgagcccgccagcatcagctgcaggagcagccagagcctggtgcacagcaacggcaacacctacctgcactggtacctgcagaagcccggccagagcccccagctgctgatctacaaggtgagcaacaggttcagcggcgtgcccgacaggttcagcggcagcggcagcggcaccgacttcaccctgaagatcagcagggtggaggccgaggacgtgggcgtgtactactgcagccagaacacccacgtgccccccaccttcggccagggcaccaagctggagatcaagaccacgacgccagcgccgcgaccaccaacaccggcgcccaccatcgcgtcgcagcccctgtccctgcgcccagaggcgtgccggccagcggcggggggcgcagtgcacacgagggggctggacttcgcctgtgatatctacatctgggcgcccttggccgggacttgtggggtccttctcctgtcactggttatcaccctttactgcaaacggggcagaaagaaactcctgtatatattcaaacaaccatttatgagaccagtacaaactactcaagaggaagatggctgtagctgccgatttccagaagaagaagaaggaggatgtgaactgagagtgaagttcagcaggagcgcagacgcccccgcgtaccagcagggccagaaccagctctataacgagctcaatctaggacgaagagaggagtacgatgttttggacaagagacgtggccgggaccctgagatggggggaaagccgagaaggaagaaccctcaggaaggcctgtacaatgaactgcagaaagataagatggcggaggcctacagtgagattgggatgaaaggcgagcgccggaggggcaaggggcacgatggcctttaccagggtctcagtacagccaccaaggacacctacgacgcccttcacatgcaggccctgccccctcgcggcagcggcgccacaaacttctctctgctaaagcaagcaggtgatgttgaagaaaaccccgggcctatgagaatttcgaaaccacatttgagaagtatttccatccagtgctacttgtgtttacttctaaacagtcattttctaactgaagctggcattcatgtcttcattttgggctgtttcagtgcagggcttcctaaaacagaagccaactgggtgaatgtaataagtgatttgaaaaaaattgaagatcttattcaatctatgcatattgatgctactttatatacggaaagtgatgttcaccccagttgcaaagtaacagcaatgaagtgctttctcttggagttacaagttatttcacttgagtccggagatgcaagtattcatgatacagtagaaaatctgatcatcctagcaaacaacagtttgtcttctaatgggaatgtaacagaatctggatgcaaagaatgtgaggaactggaggaaaaaaatattaaagaatttttgcagagttttgtacatattgtccaaatgttcatcaacacttctggttctggcgtgaaacagactttgaattttgaccttctcaagttggcgggagacgtggagtccaacccagggcccatgagatccagtcctggcaacatggagaggattgtcatctgtctgatggtcatcttcttggggacactggtccacaaatcaagctcccaaggtcaagatcgccacatgattagaatgcgtcaacttatagatattgttgatcagctgaaaaattatgtgaatgacttggtccctgaatttctgccagctccagaagatgtagagacaaactgtgagtggtcagctttttcctgctttcagaaggcccaactaaagtcagcaaatacaggaaacaatgaaaggataatcaatgtatcaattaaaaagctgaagaggaaaccaccttccacaaatgcagggagaagacagaaacacagactaacatgcccttcatgtgattcttatgagaaaaaaccacccaaagaattcctagaaagattcaaatcacttctccaaaagatgattcatcagcatctgtcctctagaacacacggaagtgaagattcctgactgtgccttctagttgccagccatctgttgtttgcccctcccccgtgccttccttgaccctggaaggtgccactcccactgtcctttcctaataaaatgaggaaattgcatcgcattgtctgagtaggtgtcattctattctggggggtggggtggggcaggacagcaagggggaggattgggaagacaatagcaggcatgctggggatgcggtgggctctatgggaattctctagaaatattctcgaggtttaaacgtcgacgcggccgcgatatccagaaccctgaccctgccgtgtaccagctgagagactctaaatccagtgacaagtctgtctgcctattcaccgattttgattctcaaacaaatgtgtcacaaagtaaggattctgatgtgtatatcacagacaaaactgtgctagacatgaggtctatggacttcaagagcaacagtgctgtggcctggagcaacaaatctgactttgcatgtgcaaacgccttcaacaacagcattattccagaagacaccttcttccccagcccaggtaagggcagctttggtgccttcgcaggctgtttccttgcttcaggaatggccaggttctgcccagagctctggtcaatgatgtctaaaactcctctgattggtggtctcggccttatccattgcc

SEQ ID NO: 22 - protein, 824 aa, synthetic construct
  source 1..824: note = GPC3CAR-2A-IL7/15-2A-CCR19/IL21
MALPVTALLLPLALLLHAARPQVQLVQSGAEVKKPGASVKVSCKASGYTFTDYEMHWVRQAPGQGLEWMGALDPKTGDTAYSQKFKGRVTLTADKSTSTAYMELSSLTSEDTAVYYCTRFYSYTYWGQGTLVTVSSGGGGSGGGGSGGGGSDVVMTQSPLSLPVTPGEPASISCRSSQSLVHSNGNTYLHWYLQKPGQSPQLLIYKVSNRFSGVPDRFSGSGSGTDFTLKISRVEAEDVGVYYCSQNTHVPPTFGQGTKLEIKTTTPAPRPPTPAPTIASQPLSLRPEACRPAAGGAVHTRGLDFACDIYIWAPLAGTCGVLLLSLVITLYCKRGRKKLLYIFKQPFMRPVQTTQEEDGCSCRFPEEEEGGCELRVKFSRSADAPAYQQGQNQLYNELNLGRREEYDVLDKRRGRDPEMGGKPRRKNPQEGLYNELQKDKMAEAYSEIGMKGERRRGKGHDGLYQGLSTATKDTYDALHMQALPPRGSGATNFSLLKQAGDVEENPGPMFHVSFRYIFGLPPLILVLLPVASSNWVNVISDLKKIEDLIQSMHIDATLYTESDVHPSCKVTAMKCFLLELQVISLESGDASIHDTVENLIILANNSLSSNGNVTESGCKECEELEEKNIKEFLQSFVHIVQMFINTSGSGVKQTLNFDLLKLAGDVESNPGPMALLLALSLLVLWTSPAPTLSQDRHMIRMRQLIDIVDQLKNYVNDLVPEFLPAPEDVETNCEWSAFSCFQKAQLKSANTGNNERIINVSIKKLKRKPPSTNAGRRQKHRLTCPSCDSYEKKPPKEFLERFKSLLQKMIHQHLSSRTHGSEDS

SEQ ID NO: 23 - DNA, 2858 bp, synthetic construct
  source 1..2858: mol_type = other DNA; note = GPC3CAR-2A-IL7/15-2A-CCR19/IL21
ctgacctcttctcttcctcccacagggcctcgagagatctggcagcggagagggcagaggaagtcttctaacatgcggtgacgtggaggagaatcccggccctaggctcgagatggccttaccagtgaccgccttgctcctgccgctggccttgctgctccacgccgccaggccgcaggtgcagctggtgcagtctggagctgaggtgaagaagcctggggcctcagtgaaggtctcctgcaaggcttctggatacaccttcaccgactatgaaatgcactgggtgcgacaggcccctggacaagggcttgagtggatgggagctcttgatcctaaaactggtgatactgcctacagtcagaagttcaagggcagagtcacgctgaccgcggacaaatccacgagcacagcctacatggagctgagcagcctgacatctgaggacacggccgtgtattactgtacaagattctactcctatacttactggggccagggaaccctggtcaccgtctcctcaggaggaggaggctctggaggaggagggagtggaggcgggggaagcgacgtggtgatgacccagagccccctgagcctgcccgtgacccccggcgagcccgccagcatcagctgcaggagcagccagagcctggtgcacagcaacggcaacacctacctgcactggtacctgcagaagcccggccagagcccccagctgctgatctacaaggtgagcaacaggttcagcggcgtgcccgacaggttcagcggcagcggcagcggcaccgacttcaccctgaagatcagcagggtggaggccgaggacgtgggcgtgtactactgcagccagaacacccacgtgccccccaccttcggccagggcaccaagctggagatcaagaccacgacgccagcgccgcgaccaccaacaccggcgcccaccatcgcgtcgcagcccctgtccctgcgcccagaggcgtgccggccagcggcggggggcgcagtgcacacgagggggctggacttcgcctgtgatatctacatctgggcgcccttggccgggacttgtggggtccttctcctgtcactggttatcaccctttactgcaaacggggcagaaagaaactcctgtatatattcaaacaaccatttatgagaccagtacaaactactcaagaggaagatggctgtagctgccgatttccagaagaagaagaaggaggatgtgaactgagagtgaagttcagcaggagcgcagacgcccccgcgtaccagcagggccagaaccagctctataacgagctcaatctaggacgaagagaggagtacgatgttttggacaagagacgtggccgggaccctgagatggggggaaagccgagaaggaagaaccctcaggaaggcctgtacaatgaactgcagaaagataagatggcggaggcctacagtgagattgggatgaaaggcgagcgccggaggggcaaggggcacgatggcctttaccagggtctcagtacagccaccaaggacacctacgacgcccttcacatgcaggccctgccccctcgcggcagcggcgccacaaacttctctctgctaaagcaagcaggtgatgttgaagaaaaccccgggcctatgttccatgtttcttttaggtatatctttggacttcctcccctgatccttgttctgttgccagtagcatcatctaactgggtgaatgtaataagtgatttgaaaaaaattgaagatcttattcaatctatgcatattgatgctactttatatacggaaagtgatgttcaccccagttgcaaagtaacagcaatgaagtgctttctcttggagttacaagttatttcacttgagtccggagatgcaagtattcatgatacagtagaaaatctgatcatcctagcaaacaacagtttgtcttctaatgggaatgtaacagaatctggatgcaaagaatgtgaggaactggaggaaaaaaatattaaagaatttttgcagagttttgtacatattgtccaaatgttcatcaacacttctggttctggcgtgaaacagactttgaattttgaccttctcaagttggcgggagacgtggagtccaacccagggcccatggccctgctactggccctcagcctgctggttctctggacttccccagccccaactctgagtcaagatcgccacatgattagaatgcgtcaacttatagatattgttgatcagctgaaaaattatgtgaatgacttggtccctgaatttctgccagctccagaagatgtagagacaaactgtgagtggtcagctttttcctgctttcagaaggcccaactaaagtcagcaaatacaggaaacaatgaaaggataatcaatgtatcaattaaaaagctgaagaggaaaccaccttccacaaatgcagggagaagacagaaacacagactaacatgcccttcatgtgattcttatgagaaaaaaccacccaaagaattcctagaaagattcaaatcacttctccaaaagatgattcatcagcatctgtcctctagaacacacggaagtgaagattcctgactgtgccttctagttgccagccatctgttgtttgcccctcccccgtgccttccttgaccctggaaggtgccactcccactgtcctttcctaataaaatgaggaaattgcatcgcattgtctgagtaggtgtcattctattctggggggtggggtggggcaggacagcaagggggaggattgggaagacaatagcaggcatgctggggatgcggtgggctctatgggaattctctagaaatattctcgaggtttaaacgtcgacgcggccgc

SEQ ID NO: 24 - DNA, 3658 bp, synthetic construct
  source 1..3658: mol_type = other DNA; note = GPC3CAR-2A-IL7/15-2A-CCR19/IL21 with homologous arms
cagtttgctttgctgggcctttttcccatgcctgcctttactctgccagagttatattgctggggttttgaagaagatcctattaaataaaagaataagcagtattattaagtagccctgcatttcaggtttccttgagtggcaggccaggcctggccgtgaacgttcactgaaatcatggcctcttggccaagattgatagcttgtgcctgtccctgagtcccagtccatcacgagcagctggtttctaagatgctatttcccgtataaagcatgagaccgtgacttgccagccccacagagccccgcccttgtccatcactggcatctggactccagcctgggttggggcaaagagggaaatgagatcatgtcctaaccctgatcctcttgtcccacactgacctcttctcttcctcccacagggcctcgagagatctggcagcggagagggcagaggaagtcttctaacatgcggtgacgtggaggagaatcccggccctaggctcgagatggccttaccagtgaccgccttgctcctgccgctggccttgctgctccacgccgccaggccgcaggtgcagctggtgcagtctggagctgaggtgaagaagcctggggcctcagtgaaggtctcctgcaaggcttctggatacaccttcaccgactatgaaatgcactgggtgcgacaggcccctggacaagggcttgagtggatgggagctcttgatcctaaaactggtgatactgcctacagtcagaagttcaagggcagagtcacgctgaccgcggacaaatccacgagcacagcctacatggagctgagcagcctgacatctgaggacacggccgtgtattactgtacaagattctactcctatacttactggggccagggaaccctggtcaccgtctcctcaggaggaggaggctctggaggaggagggagtggaggcgggggaagcgacgtggtgatgacccagagccccctgagcctgcccgtgacccccggcgagcccgccagcatcagctgcaggagcagccagagcctggtgcacagcaacggcaacacctacctgcactggtacctgcagaagcccggccagagcccccagctgctgatctacaaggtgagcaacaggttcagcggcgtgcccgacaggttcagcggcagcggcagcggcaccgacttcaccctgaagatcagcagggtggaggccgaggacgtgggcgtgtactactgcagccagaacacccacgtgccccccaccttcggccagggcaccaagctggagatcaagaccacgacgccagcgccgcgaccaccaacaccggcgcccaccatcgcgtcgcagcccctgtccctgcgcccagaggcgtgccggccagcggcggggggcgcagtgcacacgagggggctggacttcgcctgtgatatctacatctgggcgcccttggccgggacttgtggggtccttctcctgtcactggttatcaccctttactgcaaacggggcagaaagaaactcctgtatatattcaaacaaccatttatgagaccagtacaaactactcaagaggaagatggctgtagctgccgatttccagaagaagaagaaggaggatgtgaactgagagtgaagttcagcaggagcgcagacgcccccgcgtaccagcagggccagaaccagctctataacgagctcaatctaggacgaagagaggagtacgatgttttggacaagagacgtggccgggaccctgagatggggggaaagccgagaaggaagaaccctcaggaaggcctgtacaatgaactgcagaaagataagatggcggaggcctacagtgagattgggatgaaaggcgagcgccggaggggcaaggggcacgatggcctttaccagggtctcagtacagccaccaaggacacctacgacgcccttcacatgcaggccctgccccctcgcggcagcggcgccacaaacttctctctgctaaagcaagcaggtgatgttgaagaaaaccccgggcctatgttccatgtttcttttaggtatatctttggacttcctcccctgatccttgttctgttgccagtagcatcatctaactgggtgaatgtaataagtgatttgaaaaaaattgaagatcttattcaatctatgcatattgatgctactttatatacggaaagtgatgttcaccccagttgcaaagtaacagcaatgaagtgctttctcttggagttacaagttatttcacttgagtccggagatgcaagtattcatgatacagtagaaaatctgatcatcctagcaaacaacagtttgtcttctaatgggaatgtaacagaatctggatgcaaagaatgtgaggaactggaggaaaaaaatattaaagaatttttgcagagttttgtacatattgtccaaatgttcatcaacacttctggttctggcgtgaaacagactttgaattttgaccttctcaagttggcgggagacgtggagtccaacccagggcccatggccctgctactggccctcagcctgctggttctctggacttccccagccccaactctgagtcaagatcgccacatgattagaatgcgtcaacttatagatattgttgatcagctgaaaaattatgtgaatgacttggtccctgaatttctgccagctccagaagatgtagagacaaactgtgagtggtcagctttttcctgctttcagaaggcccaactaaagtcagcaaatacaggaaacaatgaaaggataatcaatgtatcaattaaaaagctgaagaggaaaccaccttccacaaatgcagggagaagacagaaacacagactaacatgcccttcatgtgattcttatgagaaaaaaccacccaaagaattcctagaaagattcaaatcacttctccaaaagatgattcatcagcatctgtcctctagaacacacggaagtgaagattcctgactgtgccttctagttgccagccatctgttgtttgcccctcccccgtgccttccttgaccctggaaggtgccactcccactgtcctttcctaataaaatgaggaaattgcatcgcattgtctgagtaggtgtcattctattctggggggtggggtggggcaggacagcaagggggaggattgggaagacaatagcaggcatgctggggatgcggtgggctctatgggaattctctagaaatattctcgaggtttaaacgtcgacgcggccgcgatatccagaaccctgaccctgccgtgtaccagctgagagactctaaatccagtgacaagtctgtctgcctattcaccgattttgattctcaaacaaatgtgtcacaaagtaaggattctgatgtgtatatcacagacaaaactgtgctagacatgaggtctatggacttcaagagcaacagtgctgtggcctggagcaacaaatctgactttgcatgtgcaaacgccttcaacaacagcattattccagaagacaccttcttccccagcccaggtaagggcagctttggtgccttcgcaggctgtttccttgcttcaggaatggccaggttctgcccagagctctggtcaatgatgtctaaaactcctctgattggtggtctcggccttatccattgcc

SEQ ID NO: 25 - DNA, 20 bp, synthetic construct
  source 1..20: mol_type = other DNA; note = sgRNA trageting TRAC
tcagggttctggatatctgt

SEQ ID NO: 26 - DNA, 514 bp, synthetic construct
  source 1..514: mol_type = other DNA; note = PGK promoter
ttggggttgcgccttttccaaggcagccctgggtttgcgcagggacgcggctgctctgggcgtggttccgggaaacgcagcggcgccgaccctgggtctcgcacattcttcacgtccgttcgcagcgtcacccggatcttcgccgctacccttgtgggccccccggcgacgcttcctgctccgcccctaagtcgggaaggttccttgcggttcgcggcgtgccggacgtgacaaacggaagccgcacgtctcactagtaccctcgcagacggacagcgccagggagcaatggcagcgcgccgaccgcgatgggctgtggccaatagcggctgctcagcagggcgcgccgagagcagcggccgggaaggggcggtgcgggaggcggggtgtggggcggtagtgtgggccctgttcctgcccgcgcggtgttccgcattctgcaagcctccggagcgcacgtcggcagtcggctccctcgttgaccgaatcaccgacctctctccccagggggatc

SEQ ID NO: 27 - DNA, 4267 bp, synthetic construct
  source 1..4267: mol_type = other DNA; note = BCMA CAR-2A-IL15 with homologous arms
cagtttgctttgctgggcctttttcccatgcctgcctttactctgccagagttatattgctggggttttgaagaagatcctattaaataaaagaataagcagtattattaagtagccctgcatttcaggtttccttgagtggcaggccaggcctggccgtgaacgttcactgaaatcatggcctcttggccaagattgatagcttgtgcctgtccctgagtcccagtccatcacgagcagctggtttctaagatgctatttcccgtataaagcatgagaccgtgacttgccagccccacagagccccgcccttgtccatcactggcatctggactccagcctgggttggggcaaagagggaaatgagatcatgtcctaaccctgatcctcttgtcccacactgacctcttctcttcctcccacagggcctcgagagatctggcagcggagagggcagaggaagtcttctaacatgcggtgacgtggaggagaatcccggccctaggctcgagatggccttaccagtgaccgccttgctcctgccgctggccttgctgctccacgccgccaggccgcaggtgcagctggtgcagagcggcgccgaggtgaagaagcccggcgccagcgtgaaggtgagctgcaaggccagcggctacagcttccccgactactacatcaactgggtgaggcaggcccccggccagggcctggagtggatgggctggatctacttcgccagcggcaacagcgagtacaaccagaagttcaccggcagggtgaccatgaccagggacaccagcatcaacaccgcctacatggagctgagcagcctgaccagcgaggacaccgccgtgtacttctgcgccagcctgtacgactacgactggtacttcgacgtgtggggccagggcaccatggtgaccgtgagcagcggaggaggaggctctggaggaggagggagtggaggcgggggaagcgacatcgtgatgacccagacccccctgagcctgagcgtgacccccggccagcccgccagcatcagctgcaagagcagccagagcctggtgcacagcaacggcaacacctacctgcactggtacctgcagaagcccggccagagcccccagctgctgatctacaaggtgagcaacaggttcagcggcgtgcccgacaggttcagcggcagcggcagcggcaccgacttcaccctgaagatcagcagggtggaggccgaggacgtgggcatctactactgcagccagagcagcatctacccctggaccttcggccagggcaccaagctggagatcaagaccacgacgccagcgccgcgaccaccaacaccggcgcccaccatcgcgtcgcagcccctgtccctgcgcccagaggcgtgccggccagcggcggggggcgcagtgcacacgagggggctggacttcgcctgtgatatctacatctgggcgcccttggccgggacttgtggggtccttctcctgtcactggttatcaccctttactgcaaacggggcagaaagaaactcctgtatatattcaaacaaccatttatgagaccagtacaaactactcaagaggaagatggctgtagctgccgatttccagaagaagaagaaggaggatgtgaactgagagtgaagttcagcaggagcgcagacgcccccgcgtaccagcagggccagaaccagctctataacgagctcaatctaggacgaagagaggagtacgatgttttggacaagagacgtggccgggaccctgagatggggggaaagccgagaaggaagaaccctcaggaaggcctgtacaatgaactgcagaaagataagatggcggaggcctacagtgagattgggatgaaaggcgagcgccggaggggcaaggggcacgatggcctttaccagggtctcagtacagccaccaaggacacctacgacgcccttcacatgcaggccctgccccctcgcggcagcggcgccacaaacttctctctgctaaagcaagcaggtgatgttgaagaaaaccccgggcctatgctggtccgcaggggcgcgcgcgcagggcccaggatgccgcggggctggaccgcgctttgcttgctgagtttgctgccttctgggttcatgagtcttgacaacaacggtactgctaccccagagttacctacccagggaacattttcaaatgtttctacaaatgtatcctaccaagaaactacaacacctagtacccttggaagtaccagcctgcaccctgtgtctcaacatggcaatgaggccacaacaaacatcacagaaacgacagtcaaattcacatctacctctgtgataacctcagtttatggaaacacaaactcttctgtccagtcacagacctctgtaatcagcacagtgttcaccaccccagccaacgtttcaactccagagacaaccttgaagcctagcctgtcacctggaaatgtttcagacctttcaaccactagcactagccttgcaacatctcccactaaaccctatacatcatcttctcctatcctaagtgacatcaaggcagaaatcaaatgttcaggcatcagagaagtgaaattgactcagggcatctgcctggagcaaaataagacctccagctgtgcggagtttaagaaggacaggggagagggcctggcccgagtgctgtgtggggaggagcaggctgatgctgatgctggggcccaggtatgctccctgctccttgcccagtctgaggtgaggcctcagtgtctactgctggtcttggccaacagaacagaaatttccagcaaactccaacttatgaaaaagcaccaatctgacctgaaaaagctggggatcctagatttcactgagcaagatgttgcaagccaccagagctattcccaaaagaccctgattgcactggtcacctcgggagccctgctggctgtcttgggcatcactggctatttcctgatgaatcgccgcagctggagccccacaggagaaaggctggaactggagcctggttctggcgtgaaacagactttgaattttgaccttctcaagttggcgggagacgtggagtccaacccagggcccatgagaatttcgaaaccacatttgagaagtatttccatccagtgctacttgtgtttacttctaaacagtcattttctaactgaagctggcattcatgtcttcattttgggctgtttcagtgcagggcttcctaaaacagaagccaactgggtgaatgtaataagtgatttgaaaaaaattgaagatcttattcaatctatgcatattgatgctactttatatacggaaagtgatgttcaccccagttgcaaagtaacagcaatgaagtgctttctcttggagttacaagttatttcacttgagtccggagatgcaagtattcatgatacagtagaaaatctgatcatcctagcaaacaacagtttgtcttctaatgggaatgtaacagaatctggatgcaaagaatgtgaggaactggaggaaaaaaatattaaagaatttttgcagagttttgtacatattgtccaaatgttcatcaacacttcttgactgtgccttctagttgccagccatctgttgtttgcccctcccccgtgccttccttgaccctggaaggtgccactcccactgtcctttcctaataaaatgaggaaattgcatcgcattgtctgagtaggtgtcattctattctggggggtggggtggggcaggacagcaagggggaggattgggaagacaatagcaggcatgctggggatgcggtgggctctatgggaattctctagaaatattctcgaggtttaaacgtcgacgcggccgcgatatccagaaccctgaccctgccgtgtaccagctgagagactctaaatccagtgacaagtctgtctgcctattcaccgattttgattctcaaacaaatgtgtcacaaagtaaggattctgatgtgtatatcacagacaaaactgtgctagacatgaggtctatggacttcaagagcaacagtgctgtggcctggagcaacaaatctgactttgcatgtgcaaacgccttcaacaacagcattattccagaagacaccttcttccccagcccaggtaagggcagctttggtgccttcgcaggctgtttccttgcttcaggaatggccaggttctgcccagagctctggtcaatgatgtctaaaactcctctgattggtggtctcggccttatccattgcc

SEQ ID NO: 28 - DNA, 4822 bp, synthetic construct
  source 1..4822: mol_type = other DNA; note = BCMA CAR-2A-IL15-IL21 with homologous arms
cagtttgctttgctgggcctttttcccatgcctgcctttactctgccagagttatattgctggggttttgaagaagatcctattaaataaaagaataagcagtattattaagtagccctgcatttcaggtttccttgagtggcaggccaggcctggccgtgaacgttcactgaaatcatggcctcttggccaagattgatagcttgtgcctgtccctgagtcccagtccatcacgagcagctggtttctaagatgctatttcccgtataaagcatgagaccgtgacttgccagccccacagagccccgcccttgtccatcactggcatctggactccagcctgggttggggcaaagagggaaatgagatcatgtcctaaccctgatcctcttgtcccacactgacctcttctcttcctcccacagggcctcgagagatctggcagcggagagggcagaggaagtcttctaacatgcggtgacgtggaggagaatcccggccctaggctcgagatggccttaccagtgaccgccttgctcctgccgctggccttgctgctccacgccgccaggccgcaggtgcagctggtgcagagcggcgccgaggtgaagaagcccggcgccagcgtgaaggtgagctgcaaggccagcggctacagcttccccgactactacatcaactgggtgaggcaggcccccggccagggcctggagtggatgggctggatctacttcgccagcggcaacagcgagtacaaccagaagttcaccggcagggtgaccatgaccagggacaccagcatcaacaccgcctacatggagctgagcagcctgaccagcgaggacaccgccgtgtacttctgcgccagcctgtacgactacgactggtacttcgacgtgtggggccagggcaccatggtgaccgtgagcagcggaggaggaggctctggaggaggagggagtggaggcgggggaagcgacatcgtgatgacccagacccccctgagcctgagcgtgacccccggccagcccgccagcatcagctgcaagagcagccagagcctggtgcacagcaacggcaacacctacctgcactggtacctgcagaagcccggccagagcccccagctgctgatctacaaggtgagcaacaggttcagcggcgtgcccgacaggttcagcggcagcggcagcggcaccgacttcaccctgaagatcagcagggtggaggccgaggacgtgggcatctactactgcagccagagcagcatctacccctggaccttcggccagggcaccaagctggagatcaagaccacgacgccagcgccgcgaccaccaacaccggcgcccaccatcgcgtcgcagcccctgtccctgcgcccagaggcgtgccggccagcggcggggggcgcagtgcacacgagggggctggacttcgcctgtgatatctacatctgggcgcccttggccgggacttgtggggtccttctcctgtcactggttatcaccctttactgcaaacggggcagaaagaaactcctgtatatattcaaacaaccatttatgagaccagtacaaactactcaagaggaagatggctgtagctgccgatttccagaagaagaagaaggaggatgtgaactgagagtgaagttcagcaggagcgcagacgcccccgcgtaccagcagggccagaaccagctctataacgagctcaatctaggacgaagagaggagtacgatgttttggacaagagacgtggccgggaccctgagatggggggaaagccgagaaggaagaaccctcaggaaggcctgtacaatgaactgcagaaagataagatggcggaggcctacagtgagattgggatgaaaggcgagcgccggaggggcaaggggcacgatggcctttaccagggtctcagtacagccaccaaggacacctacgacgcccttcacatgcaggccctgccccctcgcggcagcggcgccacaaacttctctctgctaaagcaagcaggtgatgttgaagaaaaccccgggcctatgctggtccgcaggggcgcgcgcgcagggcccaggatgccgcggggctggaccgcgctttgcttgctgagtttgctgccttctgggttcatgagtcttgacaacaacggtactgctaccccagagttacctacccagggaacattttcaaatgtttctacaaatgtatcctaccaagaaactacaacacctagtacccttggaagtaccagcctgcaccctgtgtctcaacatggcaatgaggccacaacaaacatcacagaaacgacagtcaaattcacatctacctctgtgataacctcagtttatggaaacacaaactcttctgtccagtcacagacctctgtaatcagcacagtgttcaccaccccagccaacgtttcaactccagagacaaccttgaagcctagcctgtcacctggaaatgtttcagacctttcaaccactagcactagccttgcaacatctcccactaaaccctatacatcatcttctcctatcctaagtgacatcaaggcagaaatcaaatgttcaggcatcagagaagtgaaattgactcagggcatctgcctggagcaaaataagacctccagctgtgcggagtttaagaaggacaggggagagggcctggcccgagtgctgtgtggggaggagcaggctgatgctgatgctggggcccaggtatgctccctgctccttgcccagtctgaggtgaggcctcagtgtctactgctggtcttggccaacagaacagaaatttccagcaaactccaacttatgaaaaagcaccaatctgacctgaaaaagctggggatcctagatttcactgagcaagatgttgcaagccaccagagctattcccaaaagaccctgattgcactggtcacctcgggagccctgctggctgtcttgggcatcactggctatttcctgatgaatcgccgcagctggagccccacaggagaaaggctggaactggagcctggttctggcgtgaaacagactttgaattttgaccttctcaagttggcgggagacgtggagtccaacccagggcccatgagaatttcgaaaccacatttgagaagtatttccatccagtgctacttgtgtttacttctaaacagtcattttctaactgaagctggcattcatgtcttcattttgggctgtttcagtgcagggcttcctaaaacagaagccaactgggtgaatgtaataagtgatttgaaaaaaattgaagatcttattcaatctatgcatattgatgctactttatatacggaaagtgatgttcaccccagttgcaaagtaacagcaatgaagtgctttctcttggagttacaagttatttcacttgagtccggagatgcaagtattcatgatacagtagaaaatctgatcatcctagcaaacaacagtttgtcttctaatgggaatgtaacagaatctggatgcaaagaatgtgaggaactggaggaaaaaaatattaaagaatttttgcagagttttgtacatattgtccaaatgttcatcaacacttctggaagcggacagtgtactaattatgctctcttgaaattggctggagatgttgagagcaaccctggacctatgagatccagtcctggcaacatggagaggattgtcatctgtctgatggtcatcttcttggggacactggtccacaaatcaagctcccaaggtcaagatcgccacatgattagaatgcgtcaacttatagatattgttgatcagctgaaaaattatgtgaatgacttggtccctgaatttctgccagctccagaagatgtagagacaaactgtgagtggtcagctttttcctgctttcagaaggcccaactaaagtcagcaaatacaggaaacaatgaaaggataatcaatgtatcaattaaaaagctgaagaggaaaccaccttccacaaatgcagggagaagacagaaacacagactaacatgcccttcatgtgattcttatgagaaaaaaccacccaaagaattcctagaaagattcaaatcacttctccaaaagatgattcatcagcatctgtcctctagaacacacggaagtgaagattcctgactgtgccttctagttgccagccatctgttgtttgcccctcccccgtgccttccttgaccctggaaggtgccactcccactgtcctttcctaataaaatgaggaaattgcatcgcattgtctgagtaggtgtcattctattctggggggtggggtggggcaggacagcaagggggaggattgggaagacaatagcaggcatgctggggatgcggtgggctctatgggaattctctagaaatattctcgaggtttaaacgtcgacgcggccgcgatatccagaaccctgaccctgccgtgtaccagctgagagactctaaatccagtgacaagtctgtctgcctattcaccgattttgattctcaaacaaatgtgtcacaaagtaaggattctgatgtgtatatcacagacaaaactgtgctagacatgaggtctatggacttcaagagcaacagtgctgtggcctggagcaacaaatctgactttgcatgtgcaaacgccttcaacaacagcattattccagaagacaccttcttccccagcccaggtaagggcagctttggtgccttcgcaggctgtttccttgcttcaggaatggccaggttctgcccagagctctggtcaatgatgtctaaaactcctctgattggtggtctcggccttatccattgcc

SEQ ID NO: 29 - DNA, 5224 bp, synthetic construct
  source 1..5224: mol_type = other DNA; note = PGK-BCMA CAR-2A-IL15-IL21 with homologous arms
cagtttgctttgctgggcctttttcccatgcctgcctttactctgccagagttatattgctggggttttgaagaagatcctattaaataaaagaataagcagtattattaagtagccctgcatttcaggtttccttgagtggcaggccaggcctggccgtgaacgttcactgaaatcatggcctcttggccaagattgatagcttgtgcctgtccctgagtcccagtccatcacgagcagctggtttctaagatgctatttcccgtataaagcatgagaccgtgacttgccagccccacagagccccgcccttgtccatcactggcatctggactccagcctgggttggggcaaagagggaaatgagatcatgtcctaaccctgatcctcttgtcccacattggggttgcgccttttccaaggcagccctgggtttgcgcagggacgcggctgctctgggcgtggttccgggaaacgcagcggcgccgaccctgggtctcgcacattcttcacgtccgttcgcagcgtcacccggatcttcgccgctacccttgtgggccccccggcgacgcttcctgctccgcccctaagtcgggaaggttccttgcggttcgcggcgtgccggacgtgacaaacggaagccgcacgtctcactagtaccctcgcagacggacagcgccagggagcaatggcagcgcgccgaccgcgatgggctgtggccaatagcggctgctcagcagggcgcgccgagagcagcggccgggaaggggcggtgcgggaggcggggtgtggggcggtagtgtgggccctgttcctgcccgcgcggtgttccgcattctgcaagcctccggagcgcacgtcggcagtcggctccctcgttgaccgaatcaccgacctctctccccagggggatcatggccttaccagtgaccgccttgctcctgccgctggccttgctgctccacgccgccaggccgcaggtgcagctggtgcagagcggcgccgaggtgaagaagcccggcgccagcgtgaaggtgagctgcaaggccagcggctacagcttccccgactactacatcaactgggtgaggcaggcccccggccagggcctggagtggatgggctggatctacttcgccagcggcaacagcgagtacaaccagaagttcaccggcagggtgaccatgaccagggacaccagcatcaacaccgcctacatggagctgagcagcctgaccagcgaggacaccgccgtgtacttctgcgccagcctgtacgactacgactggtacttcgacgtgtggggccagggcaccatggtgaccgtgagcagcggaggaggaggctctggaggaggagggagtggaggcgggggaagcgacatcgtgatgacccagacccccctgagcctgagcgtgacccccggccagcccgccagcatcagctgcaagagcagccagagcctggtgcacagcaacggcaacacctacctgcactggtacctgcagaagcccggccagagcccccagctgctgatctacaaggtgagcaacaggttcagcggcgtgcccgacaggttcagcggcagcggcagcggcaccgacttcaccctgaagatcagcagggtggaggccgaggacgtgggcatctactactgcagccagagcagcatctacccctggaccttcggccagggcaccaagctggagatcaagaccacgacgccagcgccgcgaccaccaacaccggcgcccaccatcgcgtcgcagcccctgtccctgcgcccagaggcgtgccggccagcggcggggggcgcagtgcacacgagggggctggacttcgcctgtgatatctacatctgggcgcccttggccgggacttgtggggtccttctcctgtcactggttatcaccctttactgcaaacggggcagaaagaaactcctgtatatattcaaacaaccatttatgagaccagtacaaactactcaagaggaagatggctgtagctgccgatttccagaagaagaagaaggaggatgtgaactgagagtgaagttcagcaggagcgcagacgcccccgcgtaccagcagggccagaaccagctctataacgagctcaatctaggacgaagagaggagtacgatgttttggacaagagacgtggccgggaccctgagatggggggaaagccgagaaggaagaaccctcaggaaggcctgtacaatgaactgcagaaagataagatggcggaggcctacagtgagattgggatgaaaggcgagcgccggaggggcaaggggcacgatggcctttaccagggtctcagtacagccaccaaggacacctacgacgcccttcacatgcaggccctgccccctcgcggcagcggcgccacaaacttctctctgctaaagcaagcaggtgatgttgaagaaaaccccgggcctatgctggtccgcaggggcgcgcgcgcagggcccaggatgccgcggggctggaccgcgctttgcttgctgagtttgctgccttctgggttcatgagtcttgacaacaacggtactgctaccccagagttacctacccagggaacattttcaaatgtttctacaaatgtatcctaccaagaaactacaacacctagtacccttggaagtaccagcctgcaccctgtgtctcaacatggcaatgaggccacaacaaacatcacagaaacgacagtcaaattcacatctacctctgtgataacctcagtttatggaaacacaaactcttctgtccagtcacagacctctgtaatcagcacagtgttcaccaccccagccaacgtttcaactccagagacaaccttgaagcctagcctgtcacctggaaatgtttcagacctttcaaccactagcactagccttgcaacatctcccactaaaccctatacatcatcttctcctatcctaagtgacatcaaggcagaaatcaaatgttcaggcatcagagaagtgaaattgactcagggcatctgcctggagcaaaataagacctccagctgtgcggagtttaagaaggacaggggagagggcctggcccgagtgctgtgtggggaggagcaggctgatgctgatgctggggcccaggtatgctccctgctccttgcccagtctgaggtgaggcctcagtgtctactgctggtcttggccaacagaacagaaatttccagcaaactccaacttatgaaaaagcaccaatctgacctgaaaaagctggggatcctagatttcactgagcaagatgttgcaagccaccagagctattcccaaaagaccctgattgcactggtcacctcgggagccctgctggctgtcttgggcatcactggctatttcctgatgaatcgccgcagctggagccccacaggagaaaggctggaactggagcctggttctggcgtgaaacagactttgaattttgaccttctcaagttggcgggagacgtggagtccaacccagggcccatgagaatttcgaaaccacatttgagaagtatttccatccagtgctacttgtgtttacttctaaacagtcattttctaactgaagctggcattcatgtcttcattttgggctgtttcagtgcagggcttcctaaaacagaagccaactgggtgaatgtaataagtgatttgaaaaaaattgaagatcttattcaatctatgcatattgatgctactttatatacggaaagtgatgttcaccccagttgcaaagtaacagcaatgaagtgctttctcttggagttacaagttatttcacttgagtccggagatgcaagtattcatgatacagtagaaaatctgatcatcctagcaaacaacagtttgtcttctaatgggaatgtaacagaatctggatgcaaagaatgtgaggaactggaggaaaaaaatattaaagaatttttgcagagttttgtacatattgtccaaatgttcatcaacacttctggaagcggacagtgtactaattatgctctcttgaaattggctggagatgttgagagcaaccctggacctatgagatccagtcctggcaacatggagaggattgtcatctgtctgatggtcatcttcttggggacactggtccacaaatcaagctcccaaggtcaagatcgccacatgattagaatgcgtcaacttatagatattgttgatcagctgaaaaattatgtgaatgacttggtccctgaatttctgccagctccagaagatgtagagacaaactgtgagtggtcagctttttcctgctttcagaaggcccaactaaagtcagcaaatacaggaaacaatgaaaggataatcaatgtatcaattaaaaagctgaagaggaaaccaccttccacaaatgcagggagaagacagaaacacagactaacatgcccttcatgtgattcttatgagaaaaaaccacccaaagaattcctagaaagattcaaatcacttctccaaaagatgattcatcagcatctgtcctctagaacacacggaagtgaagattcctgactgtgccttctagttgccagccatctgttgtttgcccctcccccgtgccttccttgaccctggaaggtgccactcccactgtcctttcctaataaaatgaggaaattgcatcgcattgtctgagtaggtgtcattctattctggggggtggggtggggcaggacagcaagggggaggattgggaagacaatagcaggcatgctggggatgcggtgggctctatgggaattctctagaaatattctcgaggtttaaacgtcgacgcggccgcgatatccagaaccctgaccctgccgtgtaccagctgagagactctaaatccagtgacaagtctgtctgcctattcaccgattttgattctcaaacaaatgtgtcacaaagtaaggattctgatgtgtatatcacagacaaaactgtgctagacatgaggtctatggacttcaagagcaacagtgctgtggcctggagcaacaaatctgactttgcatgtgcaaacgccttcaacaacagcattattccagaagacaccttcttccccagcccaggtaagggcagctttggtgccttcgcaggctgtttccttgcttcaggaatggccaggttctgcccagagctctggtcaatgatgtctaaaactcctctgattggtggtctcggccttatccattgcc

SEQ ID NO: 30 - DNA, 4159 bp, synthetic construct
  source 1..4159: mol_type = other DNA; note = PGK-GPC3 CAR-2A-IL15-2A-IL21 with homologous arms
cagtttgctttgctgggcctttttcccatgcctgcctttactctgccagagttatattgctggggttttgaagaagatcctattaaataaaagaataagcagtattattaagtagccctgcatttcaggtttccttgagtggcaggccaggcctggccgtgaacgttcactgaaatcatggcctcttggccaagattgatagcttgtgcctgtccctgagtcccagtccatcacgagcagctggtttctaagatgctatttcccgtataaagcatgagaccgtgacttgccagccccacagagccccgcccttgtccatcactggcatctggactccagcctgggttggggcaaagagggaaatgagatcatgtcctaaccctgatcctcttgtcccacattggggttgcgccttttccaaggcagccctgggtttgcgcagggacgcggctgctctgggcgtggttccgggaaacgcagcggcgccgaccctgggtctcgcacattcttcacgtccgttcgcagcgtcacccggatcttcgccgctacccttgtgggccccccggcgacgcttcctgctccgcccctaagtcgggaaggttccttgcggttcgcggcgtgccggacgtgacaaacggaagccgcacgtctcactagtaccctcgcagacggacagcgccagggagcaatggcagcgcgccgaccgcgatgggctgtggccaatagcggctgctcagcagggcgcgccgagagcagcggccgggaaggggcggtgcgggaggcggggtgtggggcggtagtgtgggccctgttcctgcccgcgcggtgttccgcattctgcaagcctccggagcgcacgtcggcagtcggctccctcgttgaccgaatcaccgacctctctccccagggggatcatggccttaccagtgaccgccttgctcctgccgctggccttgctgctccacgccgccaggccgcaggtgcagctggtgcagtctggagctgaggtgaagaagcctggggcctcagtgaaggtctcctgcaaggcttctggatacaccttcaccgactatgaaatgcactgggtgcgacaggcccctggacaagggcttgagtggatgggagctcttgatcctaaaactggtgatactgcctacagtcagaagttcaagggcagagtcacgctgaccgcggacaaatccacgagcacagcctacatggagctgagcagcctgacatctgaggacacggccgtgtattactgtacaagattctactcctatacttactggggccagggaaccctggtcaccgtctcctcaggaggaggaggctctggaggaggagggagtggaggcgggggaagcgacgtggtgatgacccagagccccctgagcctgcccgtgacccccggcgagcccgccagcatcagctgcaggagcagccagagcctggtgcacagcaacggcaacacctacctgcactggtacctgcagaagcccggccagagcccccagctgctgatctacaaggtgagcaacaggttcagcggcgtgcccgacaggttcagcggcagcggcagcggcaccgacttcaccctgaagatcagcagggtggaggccgaggacgtgggcgtgtactactgcagccagaacacccacgtgccccccaccttcggccagggcaccaagctggagatcaagaccacgacgccagcgccgcgaccaccaacaccggcgcccaccatcgcgtcgcagcccctgtccctgcgcccagaggcgtgccggccagcggcggggggcgcagtgcacacgagggggctggacttcgcctgtgatatctacatctgggcgcccttggccgggacttgtggggtccttctcctgtcactggttatcaccctttactgcaaacggggcagaaagaaactcctgtatatattcaaacaaccatttatgagaccagtacaaactactcaagaggaagatggctgtagctgccgatttccagaagaagaagaaggaggatgtgaactgagagtgaagttcagcaggagcgcagacgcccccgcgtaccagcagggccagaaccagctctataacgagctcaatctaggacgaagagaggagtacgatgttttggacaagagacgtggccgggaccctgagatggggggaaagccgagaaggaagaaccctcaggaaggcctgtacaatgaactgcagaaagataagatggcggaggcctacagtgagattgggatgaaaggcgagcgccggaggggcaaggggcacgatggcctttaccagggtctcagtacagccaccaaggacacctacgacgcccttcacatgcaggccctgccccctcgcggcagcggcgccacaaacttctctctgctaaagcaagcaggtgatgttgaagaaaaccccgggcctatgagaatttcgaaaccacatttgagaagtatttccatccagtgctacttgtgtttacttctaaacagtcattttctaactgaagctggcattcatgtcttcattttgggctgtttcagtgcagggcttcctaaaacagaagccaactgggtgaatgtaataagtgatttgaaaaaaattgaagatcttattcaatctatgcatattgatgctactttatatacggaaagtgatgttcaccccagttgcaaagtaacagcaatgaagtgctttctcttggagttacaagttatttcacttgagtccggagatgcaagtattcatgatacagtagaaaatctgatcatcctagcaaacaacagtttgtcttctaatgggaatgtaacagaatctggatgcaaagaatgtgaggaactggaggaaaaaaatattaaagaatttttgcagagttttgtacatattgtccaaatgttcatcaacacttctggttctggcgtgaaacagactttgaattttgaccttctcaagttggcgggagacgtggagtccaacccagggcccatgagatccagtcctggcaacatggagaggattgtcatctgtctgatggtcatcttcttggggacactggtccacaaatcaagctcccaaggtcaagatcgccacatgattagaatgcgtcaacttatagatattgttgatcagctgaaaaattatgtgaatgacttggtccctgaatttctgccagctccagaagatgtagagacaaactgtgagtggtcagctttttcctgctttcagaaggcccaactaaagtcagcaaatacaggaaacaatgaaaggataatcaatgtatcaattaaaaagctgaagaggaaaccaccttccacaaatgcagggagaagacagaaacacagactaacatgcccttcatgtgattcttatgagaaaaaaccacccaaagaattcctagaaagattcaaatcacttctccaaaagatgattcatcagcatctgtcctctagaacacacggaagtgaagattcctgactgtgccttctagttgccagccatctgttgtttgcccctcccccgtgccttccttgaccctggaaggtgccactcccactgtcctttcctaataaaatgaggaaattgcatcgcattgtctgagtaggtgtcattctattctggggggtggggtggggcaggacagcaagggggaggattgggaagacaatagcaggcatgctggggatgcggtgggctctatgggaattctctagaaatattctcgaggtttaaacgtcgacgcggccgcgatatccagaaccctgaccctgccgtgtaccagctgagagactctaaatccagtgacaagtctgtctgcctattcaccgattttgattctcaaacaaatgtgtcacaaagtaaggattctgatgtgtatatcacagacaaaactgtgctagacatgaggtctatggacttcaagagcaacagtgctgtggcctggagcaacaaatctgactttgcatgtgcaaacgccttcaacaacagcattattccagaagacaccttcttccccagcccaggtaagggcagctttggtgccttcgcaggctgtttccttgcttcaggaatggccaggttctgcccagagctctggtcaatgatgtctaaaactcctctgattggtggtctcggccttatccattgcc

SEQ ID NO: 31 - DNA, 357 bp, synthetic construct
  source 1..357: mol_type = other DNA; note = BCMA scFv VH
caggtgcagctggtgcagagcggcgccgaggtgaagaagcccggcgccagcgtgaaggtgagctgcaaggccagcggctacagcttccccgactactacatcaactgggtgaggcaggcccccggccagggcctggagtggatgggctggatctacttcgccagcggcaacagcgagtacaaccagaagttcaccggcagggtgaccatgaccagggacaccagcatcaacaccgcctacatggagctgagcagcctgaccagcgaggacaccgccgtgtacttctgcgccagcctgtacgactacgactggtacttcgacgtgtggggccagggcaccatggtgaccgtgagcagc

SEQ ID NO: 32 - DNA, 336 bp, synthetic construct
  source 1..336: mol_type = other DNA; note = BCMA scFv VL
gacatcgtgatgacccagacccccctgagcctgagcgtgacccccggccagcccgccagcatcagctgcaagagcagccagagcctggtgcacagcaacggcaacacctacctgcactggtacctgcagaagcccggccagagcccccagctgctgatctacaaggtgagcaacaggttcagcggcgtgcccgacaggttcagcggcagcggcagcggcaccgacttcaccctgaagatcagcagggtggaggccgaggacgtgggcatctactactgcagccagagcagcatctacccctggaccttcggccagggcaccaagctggagatcaag